European Patent Specification EP 3 632 467 B1, published September 27, 2023. Title: INHIBITORS OF COMPLEMENT FACTOR H. Applicant: DUKE UNIVERSITY. Application not yet assigned. The sequence listing filed with the application follows.

SEQUENCE LISTING (132 sequences)

SEQ ID NO: 1 - protein, 1231 aa, Homo sapiens
MRLLAKIICLMLWAICVAEDCNELPPRRNTEILTGSWSDQTYPEGTQAIYKCRPGYRSLGNVIMVCRKGEWVALNPLRKCQKRPCGHPGDTPFGTFTLTGGNVFEYGVKAVYTCNEGYQLLGEINYRECDTDGWTNDIPICEVVKCLPVTAPENGKIVSSAMEPDREYHFGQAVRFVCNSGYKIEGDEEMHCSDDGFWSKEKPKCVEISCKSPDVINGSPISQKIIYKENERFQYKCNMGYEYSERGDAVCTESGWRPLPSCEEKSCDNPYIPNGDYSPLRIKHRTGDEITYQCRNGFYPATRGNTAKCTSTGWIPAPRCTLKPCDYPDIKHGGLYHENMRRPYFPVAVGKYYSYYCDEHFETPSGSYWDHIHCTQDGWSPAVPCLRKCYFPYLENGYNQNYGRKFVQGKSIDVACHPGYALPKAQTTVTCMENGWSPTPRCIRVKTCSKSSIDIENGFISESQYTYALKEKAKYQCKLGYVTADGETSGSITCGKDGWSAQPTCIKSCDIPVFMNARTKNDFTWFKLNDTLDYECHDGYESNTGSTTGSIVCGYNGWSDLPICYERECELPKIDVHLVPDRKKDQYKVGEVLKFSCKPGFTIVGPNSVQCYHFGLSPDLPICKEQVQSCGPPPELLNGNVKEKTKEEYGHSEVVEYYCNPRFLMKGPNKIQCVDGEWTTLPVCIVEESTCGDIPELEHGWAQLSSPPYYYGDSVEFNCSESFTMIGHRSITCIHGVWTQLPQCVAIDKLKKCKSSNLIILEEHLKNKKEFDHNSNIRYRCRGKEGWIHTVCINGRWDPEVNCSMAQIQLCPPPPQIPNSHNMTTTLNYRDGEKVSVLCQENYLIQEGEEITCKDGRWQSIPLCVEKIPCSQPPQIEHGTINSSRSSQESYAHGTKLSYTCEGGFRISEENETTCYMGKWSSPPQCEGLPCKSPPEISHGVVAHMSDSYQYGEEVTYKCFEGFGIDGPAIAKCLGEKWSHPPSCIKTDCLSLPSFENAIPMGEKKDVYKAGEQVTYTCATYYKMDGASNVTCINSRWTGRPTCRDTSCVNPPTVQNAYIVSRQMSKYPSGERVRYQCRSPYEMFGDEEVMCLNGNWTEPPQCKDSTGKCGPPPPIDNGDITSFPLSVYAPASSVEYQCQNLYQLEGNKRITCRNGQWSEPPKCLHPCVISREIMENYNIALRWTAKQKLYSRTGESVEFVCKRGYRLSSRSHTLRTTCWDGKLEYPTCAKR

SEQ ID NO: 2 - protein, 59 aa, Homo sapiens
GKCGPPPPIDNGDITSFPLSVYAPASSVEYQCQNLYQLEGNKRITCRNGQWSEPPKCLH

SEQ ID NO: 3 - protein, 8 aa, Homo sapiens
PIDNGDIT

SEQ ID NO: 4 - protein, 120 aa, Artificial Sequence
  source: /note="Description of Artificial Sequence: Synthetic polypeptide"
LVESGGGVVQPGRSLRLSCAASGLTFSFYNFHWVRQTPGKGLEWVAGISYDATRTNYAGSVTGRFTISRDNSKKMLYLQMSSLGPQDTAVYHCARDRSDGQLHKVAFDSWGQGALVTVSS

SEQ ID NO: 5 - protein, 116 aa, Artificial Sequence
  source: /note="Description of Artificial Sequence: Synthetic polypeptide"
LVESGGGVVRPGRSLRLSCVASGFTFNAYGMHWVRQGPGKGLEWLAVISYEGKTVYYADSVKDRFTISRDNSRNTVSLHLNNLRGEDTAVYYCAKGSASAAVLQHWGQGTLVSVTS

SEQ ID NO: 6 - protein, 116 aa, Artificial Sequence
  source: /note="Description of Artificial Sequence: Synthetic polypeptide"
LVESGGGVVPPGKSLRLSCAASGFTFSLYGIHWVRQAPGKGLEWVAVISYDGNTKYYTDSVKGRFTISRDNAKNTIYLQMNSLRLDDTAVYYCAKGAANSATFDFWGRGTMVTVSS

SEQ ID NO: 7 - protein, 116 aa, Artificial Sequence; identical to SEQ ID NO: 6
  source: /note="Description of Artificial Sequence: Synthetic polypeptide"

SEQ ID NO: 8 - protein, 116 aa, Artificial Sequence; identical to SEQ ID NO: 6
  source: /note="Description of Artificial Sequence: Synthetic polypeptide"

SEQ ID NO: 9 - protein, 116 aa, Artificial Sequence; identical to SEQ ID NO: 6
  source: /note="Description of Artificial Sequence: Synthetic polypeptide"

SEQ ID NO: 10 - protein, 116 aa, Artificial Sequence
  source: /note="Description of Artificial Sequence: Synthetic polypeptide"
LVESGGGVVQPGKSLRLSCVASGFSFSTYGMHWVRQAPGKGLEWVAVMSFDGKTKYYADSVKGRFTISRDNPKNTLYLQMNSLRSEDTAVYYCAKGGAAAAVFDSWGPGILLTVSS

SEQ ID NO: 11 - protein, 116 aa, Artificial Sequence; identical to SEQ ID NO: 10
  source: /note="Description of Artificial Sequence: Synthetic polypeptide"

SEQ ID NO: 12 - protein, 116 aa, Artificial Sequence
  source: /note="Description of Artificial Sequence: Synthetic polypeptide"
LVESGGGVVQPGRSLRLSCAASGVTFSRYGMHWVRQAPGKGLEWVAVISYDEKTKYYADSVKGRFTISRDNSKNTLFLHMNRLRYEDTAVYYCAKGASSGAYFDYWGQGTLVTVSS

SEQ ID NO: 13 - protein, 116 aa, Artificial Sequence
  source: /note="Description of Artificial Sequence: Synthetic polypeptide"
LVESGGGVVQPGKSLRLSCVASGFTFSTYGMHWVRQAPGKGLEWVAVMSFDGKTKYYADSVKGRFTISRDNPKNTLYLQMNSLRSEDTAVYYCAKGGAAAAVFDSWGQGILLTVSS

SEQ ID NO: 14 - protein, 116 aa, Artificial Sequence
  source: /note="Description of Artificial Sequence: Synthetic polypeptide"
LVESGGGVVQPGKSLRLSCVASGFTFSSYGMHWVRQAPGKGLEWVAVMSFDGKTKYYADSVKGRFTISRDNPKNTLYLQMNSLRSEDTAVYYCAKGGAAAAVFDSWGQGILLTVSS

SEQ ID NO: 15 - protein, 116 aa, Artificial Sequence; identical to SEQ ID NO: 14
  source: /note="Description of Artificial Sequence: Synthetic polypeptide"

SEQ ID NO: 16 - protein, 116 aa, Artificial Sequence
  source: /note="Description of Artificial Sequence: Synthetic polypeptide"
LVESGGGVVQPGRSLRLSCAASGFTFSRYGMHWVRQAPGKGLEWVAVMSYDGSTKYYADSVKGRFAISRDNPKNTLFLQMNSLRPDDTAVYYCAKGGAAAAVMDVWGKGTTVTVSS

SEQ ID NO: 17 - protein, 116 aa, Artificial Sequence; identical to SEQ ID NO: 16
  source: /note="Description of Artificial Sequence: Synthetic polypeptide"

SEQ ID NO: 18 - protein, 121 aa, Artificial Sequence
  source: /note="Description of Artificial Sequence: Synthetic polypeptide"
EVQLVESGGGVVQPGRSLRLSCAASGFTFNRFGMHWVRQRQVPGKGLEWVAVISYDDNTKYYADSVKGRFTISRDNNKSTLYLQMSSLRVEDTAVYFCAKGSTAAAVLDYWGQGTLVTVSS

SEQ ID NO: 19 - protein, 118 aa, Artificial Sequence
  source: /note="Description of Artificial Sequence: Synthetic polypeptide"
LVESGGGLVQPGGSLRLSCAASGFTFSSYEMNWVRQAPGKGLEWVSYISSSGSTIYYADSVKGRFTISRDNAKNSLYLQMNSLRAEDTAVYYCARVEQLAPSPYMDVWGKGTTVTVSS

SEQ ID NO: 20 - protein, 124 aa, Artificial Sequence
  source: /note="Description of Artificial Sequence: Synthetic polypeptide"
QVQLVQSGAEVKKPGESLKISCKGSGYSFTSYWIGWVRQMPGKGLEWMGIIYPGDSDTRYSPSFQGQVTISADKSISTAYLQWSSLKASDTAMYYCARRGLRGAYYYYYGMDVWGQGTTVTVSS

SEQ ID NO: 21 - protein, 110 aa, Artificial Sequence
  source: /note="Description of Artificial Sequence: Synthetic polypeptide"
MTQSPDSLTLSLGERATINCRSSRTVLYRSNNKNYLAWYQHKPGQPPKLLMSWASTRETGVPDRFSGSGSGTHFTLTITSLQPEDVAVYYCQQYYSPPWTFGQGTKVEIR

SEQ ID NO: 22 - protein, 110 aa, Artificial Sequence
  source: /note="Description of Artificial Sequence: Synthetic polypeptide"
MTQSPGSLAVSLGSRATINCKSSRSLLYRSNNKNYLAWYQQKPGQSPRLLIYWASSRESGVPDRFSGGGSGTSFTLTISSLQAEDVAVYYCQQYFNPPWTFGQGTKVEIK

SEQ ID NO: 23 - protein, 110 aa, Artificial Sequence; identical to SEQ ID NO: 21
  source: /note="Description of Artificial Sequence: Synthetic polypeptide"

SEQ ID NO: 24 - protein, 110 aa, Artificial Sequence; identical to SEQ ID NO: 21
  source: /note="Description of Artificial Sequence: Synthetic polypeptide"

SEQ ID NO: 25 - protein, 110 aa, Artificial Sequence; identical to SEQ ID NO: 21
  source: /note="Description of Artificial Sequence: Synthetic polypeptide"

SEQ ID NO: 26 - protein, 110 aa, Artificial Sequence; identical to SEQ ID NO: 21
  source: /note="Description of Artificial Sequence: Synthetic polypeptide"

SEQ ID NO: 27 - protein, 110 aa, Artificial Sequence
  source: /note="Description of Artificial Sequence: Synthetic polypeptide"
MTQSPNSLAVSLGGRATINCKASQSILYRSNNKNYLAWYQHKAGQPPKLLIYWASTRESGVPERFSGSGSRTDFTLTINGLQAEDVAVYYCQQYYNPPWTFGQGTKVEIK

SEQ ID NO: 28 - protein, 110 aa, Artificial Sequence; identical to SEQ ID NO: 27
  source: /note="Description of Artificial Sequence: Synthetic polypeptide"

SEQ ID NO: 29 - protein, 110 aa, Artificial Sequence
  source: /note="Description of Artificial Sequence: Synthetic polypeptide"
MTQSPDSLAVSLGERATIKCKSSQSVLYSSNNKNYLAWYQHKPGQPPKVLVYWASTRESGVPDRFSGSGSGTDFTLTISSLQAEDVAVYYCQQYYNPPWTFGQGTKVAIK

SEQ ID NO: 30 - protein, 110 aa, Artificial Sequence
  source: /note="Description of Artificial Sequence: Synthetic polypeptide"
MTQSPNSLAVSLGGRATINCKTSQSILYRSNNKNYLAWYQHKPGQPPKLLIYWASTRESRVPDRFSGSGSRTDFTLTISGLQAEDVAVYYCQQYYNPPWTFGQGTKVEIK

SEQ ID NO: 31 - protein, 110 aa, Artificial Sequence
  source: /note="Description of Artificial Sequence: Synthetic polypeptide"
MTQSPNSLAVSLGGRATINCKTSQSILYRSNNKNYLAWYQHKSGQPPKLLIYWASTRESGVPDRFSGSGSRTDFTLTISGLQAEDVAVYYCQQYYNPPWTFGQGTKVEIK

SEQ ID NO: 32 - protein, 110 aa, Artificial Sequence; identical to SEQ ID NO: 31
  source: /note="Description of Artificial Sequence: Synthetic polypeptide"

SEQ ID NO: 33 - protein, 110 aa, Artificial Sequence
  source: /note="Description of Artificial Sequence: Synthetic polypeptide"
MTQSPDSLTVSLGERATISCKSSQRLLYSSNNKNYLAWYQQKPGQPPKLLMYWASTRESGVPDRFSGSGSGTDFSLTISSLQAEDVAVYYCQQYYNPPWTFGQGTKVEVK

SEQ ID NO: 34 - protein, 110 aa, Artificial Sequence; identical to SEQ ID NO: 33
  source: /note="Description of Artificial Sequence: Synthetic polypeptide"

SEQ ID NO: 35 - protein, 113 aa, Artificial Sequence
  source: /note="Description of Artificial Sequence: Synthetic polypeptide"
DIVMTQSPDSLTLSLGERATINCKSSQSLFYRSNNKSYLAWYQQKPGQPPKLLIYWASVRESGVPDRFTGSGSVTDFTLTISSLRAEDVAVYYCQQYFTTPLTFGGGTKVAIK

SEQ ID NO: 36 - protein, 110 aa, Artificial Sequence
  source: /note="Description of Artificial Sequence: Synthetic polypeptide"
MTQSLDSLTVSLGERATINCKSSQSLLYTSNNKNYLAWYQQKSGQPPKLLIYWASIRDSGVPDRFSGSGSATDFTLTINNLQAEDVAVYFCQQYYKTPLTFGGGTKVEVR

SEQ ID NO: 37 - protein, 107 aa, Artificial Sequence
  source: /note="Description of Artificial Sequence: Synthetic polypeptide"
  MOD_RES (4)..(4): Any amino acid
DIQXTQSPSTLSASVGDRVTITCRASQSISSWLAWYQQKPGKAPKLLIYKASSLESGVPSRFSGSGSGTEFTLTISSLQPDDFATYYCQQYNSYSWTFGQGTKVEIK

SEQ ID NO: 38 - DNA, 368 bp, Artificial Sequence
  source: /note="Description of Artificial Sequence: Synthetic polynucleotide"
gaggtgcagctggtggagtctgggggaggcgtggtccagcctgggaggtccctgagactctcctgcgcagcctctggactcaccttcagtttctataatttccactgggtccgccagactccaggcaaggggctggagtgggtggcaggcatctcatacgatgcaaccaggacgaactacgcaggctcgtcacgggccgattcaccatttccagagacaattccaagaaaatgctgtatctgcaaatgagcagcctgggacctcaagacacggctgtatatcattgtgcgagagatcgttctgacgggcaactgcataaagtggcttttgactcctggggccagggagccctggtcaccgtctcatca

SEQ ID NO: 39 - DNA, 357 bp, Artificial Sequence
  source: /note="Description of Artificial Sequence: Synthetic polynucleotide"
gaggtgcagctggtggagtctgggggaggcgtggtccggcctgggcggtccctgagactctcctgtgttgcctctggtttcaccttcaatgcttatggcatgcattgggtccgccagggtccaggcaagggccttgagtggctggcggtcatttcatatgaaggaaagactgtttattatgcagattccgttaaggaccgtttcaccatctccagagacaattccaggaacacggtgtctctacatctgaacaacctgagaggtgaggacacggctgtctattactgtgcgaaggggtcggcttcagcagcagtcctccaacactggggtcagggcaccctggtcagcgtcacgtca

SEQ ID NO: 40 - DNA, 357 bp, Artificial Sequence
  source: /note="Description of Artificial Sequence: Synthetic polynucleotide"
gaggtgcagctggtggagtctgggggaggcgtggtcccgcctgggaagtccctgagactctcctgtgcagcctctggattcaccttcagtctctatggcatacactgggtccgccaggctcccggcaagggactggagtgggtggcagttatctcatatgatggaaatactaaatactatacagactctgtaaagggtcgattcaccatctccagagacaatgccaagaacacaatttatctgcaaatgaacagtctaagacttgacgacacggctgtttattactgtgcgaaaggagcggcgaatagcgctacttttgatttctggggccgagggacaatggtcaccgtctcttca

SEQ ID NO: 41 - DNA, 357 bp, Artificial Sequence; identical to SEQ ID NO: 40
  source: /note="Description of Artificial Sequence: Synthetic polynucleotide"

SEQ ID NO: 42 - DNA, 357 bp, Artificial Sequence; identical to SEQ ID NO: 40
  source: /note="Description of Artificial Sequence: Synthetic polynucleotide"

SEQ ID NO: 43 - DNA, 357 bp, Artificial Sequence; identical to SEQ ID NO: 40
  source: /note="Description of Artificial Sequence: Synthetic polynucleotide"

SEQ ID NO: 44 - DNA, 246 bp, Artificial Sequence
  source: /note="Description of Artificial Sequence: Synthetic polynucleotide"
gaggtgcagctggtggagtctgggggaggcgtggtccagcctggaaagtctctgagactctcctgtgtagcctctggattcagcttcagtacttatggcatgcactgggtccgccaggctccaggcaaggggctggagtgggtggcggttatgtcatttgatggaaagactaaatactatgcagactccgtgaagggccgattcaccatctccagagacaatcccaagaacacactatatctgcaa

SEQ ID NO: 45 - DNA, 357 bp, Artificial Sequence
  source: /note="Description of Artificial Sequence: Synthetic polynucleotide"
gaggtgcagctggtggagtctgggggaggcgtggtccagcctggaaagtctctgagactctcctgtgtagcctctggattcagcttcagtacttatggcatgcactgggtccgccaggctccaggcaaggggctggagtgggtggcggttatgtcatttgatggaaagactaaatactatgcagactccgtgaagggccgattcaccatctccagagacaatcccaagaacacactatatctgcaaatgaacagcctgagaagcgaagacacggctgtgtattattgtgcgaaggggggtgcagcagcggccgtctttgactcctggggcccgggaatactgctcaccgtctcctca

SEQ ID NO: 46 - DNA, 357 bp, Artificial Sequence
  source: /note="Description of Artificial Sequence: Synthetic polynucleotide"
gaggtgcagctggtggagtctgggggaggcgtggtccagcctgggaggtccctaagactctcctgtgcagcctctggagtcaccttcagtagatatggcatgcactgggtccgccaggctccaggcaaggggctggagtgggtggcagttatatcatatgatgaaaagactaaatactatgcagactccgtgaagggccgattcaccatctccagagacaattccaagaacacactgtttctgcacatgaacagactgagatatgaggacacggctgtatattattgtgcgaaaggggccagtagcggtgcgtactttgactactggggccagggtaccctggtcaccgtctcctca

SEQ ID NO: 47 - DNA, 357 bp, Artificial Sequence
  source: /note="Description of Artificial Sequence: Synthetic polynucleotide"
gaggtgcagctggtggagtctgggggaggcgtggtccagcctggaaagtctctgagactctcctgtgtagcctctggattcaccttcagtacttatggcatgcactgggtccgccaggctccaggcaaggggctggagtgggtggcagttatgtcatttgatggaaagactaaatactatgcagactccgtgaagggccgattcaccatctccagagacaatcccaagaacacactatatctgcaaatgaacagcctgagaagcgaagacacggctgtgtattattgtgcgaaggggggtgcagcagcggccgtctttgactcctggggccagggaatactgctcaccgtctcctca

SEQ ID NO: 48 - DNA, 357 bp, Artificial Sequence
  source: /note="Description of Artificial Sequence: Synthetic polynucleotide"
gaggtgcagctggtggagtctgggggaggcgtggtccagcctggaaagtctctgagactctcctgtgtagcctctggattcaccttcagtagttatggcatgcactgggtccgccaggctccgggcaaggggctggagtgggtggcggttatgtcatttgatggaaagactaaatactatgcagactccgtgaagggccgattcaccatctccagagacaaccccaagaacacactatatctgcaaatgaacagcctgagaagcgaagacacggctgtctattattgtgcgaaggggggtgcagcagcggccgtctttgactcctggggccagggaatactgctcaccgtctcctca

SEQ ID NO: 49 - DNA, 357 bp, Artificial Sequence; identical to SEQ ID NO: 48
  source: /note="Description of Artificial Sequence: Synthetic polynucleotide"

SEQ ID NO: 50 - DNA, 356 bp, Artificial Sequence
  source: /note="Description of Artificial Sequence: Synthetic polynucleotide"
gaggtgcagctggtggagtctgggggaggcgtggtccagcctgggaggtccctgagactctcctgtgcagcctctggattcaccttcagtagatatggcatgcactgggtccgccaggctccaggcaaggggctggagtgggtggcagttatgtcatatgatggaagtactaaatactatgcagactccgtgaagggccgcttcgccatctccagagacaatcccaagaacacgctatttctgcaaatgaacagcctgagacctgacgacacggctgtatattactgtgcgaaagggggggcggcacagctgtcatggacgtctggggcaaagggaccacggtcaccgtctcctca

SEQ ID NO: 51 - DNA, 357 bp, Artificial Sequence
  source: /note="Description of Artificial Sequence: Synthetic polynucleotide"
gaggtgcagctggtggagtctgggggaggcgtggtccagcctgggaggtccctgagactctcctgtgcagcctctggattcaccttcagtagatatggcatgcactgggtccgccaggctccaggcaaggggctggagtgggtggcagttatgtcatatgatggaagtactaaatactatgcagactccgtgaagggccgcttcgccatctccagagacaatcccaagaacacgctatttctgcaaatgaacagcctgagacctgacgacacggctgtatattactgtgcgaaagggggggcggcagcagctgtcatggacgtctggggcaaagggaccacggtcaccgtctcctca

SEQ ID NO: 52 - DNA, 363 bp, Artificial Sequence
  source: /note="Description of Artificial Sequence: Synthetic polynucleotide"
gaggtgcagctggtggagtctgggggaggcgtggtccagcctgggaggtccctgagactctcctgtgcagcctctggattcaccttcaataggtttggcatgcactgggtccgccagcgccaggttccaggcaaggggctggagtgggtggcagttatctcatatgacgacaacactaaatattatgcggactccgtgaagggccgtttcaccatctccagagacaataacaagagcactctctatctgcaaatgagcagcctgagagttgaggacacggctgtctatttctgtgcgaaggggtcgacagcggcagctgttcttgactactggggccagggaacccttgtcaccgtctcctca

SEQ ID NO: 53 - DNA, 363 bp, Artificial Sequence
  source: /note="Description of Artificial Sequence: Synthetic polynucleotide"
gaggtgcagctggtggagtctgggggaggcttggtacagcctggagggtccctgagactctcctgtgcagcctctggattcaccttcagtagttatgaaatgaactgggtccgccaggctccagggaaggggctggagtgggtttcatacattagtagtagtggtagtaccatatactacgcagactctgtgaagggccgattcaccatctccagagacaacgccaagaactcactgtatctgcaaatgaacagcctgagagccgaggacacggctgtttattactgtgcgagagtagagcagctcgccccctccccctacatggacgtctggggcaaagggaccacggtcaccgtctcctca

SEQ ID NO: 54 - DNA, 372 bp, Artificial Sequence
  source: /note="Description of Artificial Sequence: Synthetic polynucleotide"
caggtgcagctggtgcagtctggggcagaggtgaaaaagcccggggagtctctgaagatctcctgtaagggttctggatacagctttaccagctactggatcggctgggtgcgccagatgcccgggaaaggcctggagtggatggggatcatctatcctggtgactctgataccagatacagcccgtccttccaaggccaggtcaccatctcagccgacaagtccatcagcaccgcctacctgcagtggagcagcctgaaggcctcggacaccgccatgtattactgtgcgagacggggtcttcgaggggcctactactactactacggtatggacgtctggggccaagggaccacggtcaccgtctcctca

SEQ ID NO: 55 - DNA, 339 bp, Artificial Sequence
  source: /note="Description of Artificial Sequence: Synthetic polynucleotide"
gacatcgtgatgacccagtctccagactccctgactctgtctctgggcgagagggccaccatcaactgcagatccagccggactgttttatacaggtccaacaataaaaattacttagcttggtatcaacataaaccaggacagcctcctaagttgctcatgtcctgggcatctacccgggaaaccggggtccctgaccgattcagtggcagcggttctgggacacatttcactctcaccatcaccagcctgcagcctgaagatgtggcagtttattactgtcaacagtattatagtcctccgtggacgttcggccaagggaccaaggtggaaatcaga

SEQ ID NO: 56 - DNA, 246 bp, Artificial Sequence
  source: /note="Description of Artificial Sequence: Synthetic polynucleotide"
gacatcgtgatgacccagtctccaggctccctggctgtgtctctgggctcgagggccaccatcaactgcaagtccagccggagtcttttatacaggtccaacaataagaattatttagcttggtatcaacagaaaccaggacagtctcctcggcttctcatttattgggcatcttcccgggaatccggggtccctgaccgattcagtggcggcgggtctgggacaagtttcactctcaccatcagc

SEQ ID NO: 57 - DNA, 339 bp, Artificial Sequence; identical to SEQ ID NO: 55
  source: /note="Description of Artificial Sequence: Synthetic polynucleotide"

SEQ ID NO: 58 - DNA, 339 bp, Artificial Sequence; identical to SEQ ID NO: 55
  source: /note="Description of Artificial Sequence: Synthetic polynucleotide"

SEQ ID NO: 59 - DNA, 339 bp, Artificial Sequence; identical to SEQ ID NO: 55
  source: /note="Description of Artificial Sequence: Synthetic polynucleotide"

SEQ ID NO: 60 - DNA, 339 bp, Artificial Sequence; identical to SEQ ID NO: 55
  source: /note="Description of Artificial Sequence: Synthetic polynucleotide"

SEQ ID NO: 61 - DNA, 339 bp, Artificial Sequence
  source: /note="Description of Artificial Sequence: Synthetic polynucleotide"
gacatcgtgatgacccagtctccaaactccctggctgtgtctctgggcgggagggccaccatcaactgcaaggccagccagagtattttatacaggtccaacaataagaactatttagcttggtaccaacataaagcaggacagcctcccaagctgctcatttactgggcatctacccgggaatccggggtccctgagcgattcagtggcagcgggtctaggacagatttcactctcaccatcaacggcctgcaggctgaagatgtggcagtttattactgtcagcaatattataatcctccgtggacgttcggccaagggaccaaggtggaaatcaaa

SEQ ID NO: 62 - DNA, 339 bp, Artificial Sequence; identical to SEQ ID NO: 61
  source: /note="Description of Artificial Sequence: Synthetic polynucleotide"

SEQ ID NO: 63 - DNA, 339 bp, Artificial Sequence
  source: /note="Description of Artificial Sequence: Synthetic polynucleotide"
gacatcgtgatgacccagtctccagactccctggctgtgtctctgggcgagagggccaccatcaagtgcaagtccagccagagtgtcttgtacagctccaacaataagaactacttagcttggtaccagcataaaccaggacagcctcctaaggtactcgtttactgggcatccacccgggaatccggggtccctgaccgattcagtggcagcgggtctgggacagatttcactctcaccatcagcagcctgcaggctgaagatgtggcagtttattactgtcaacaatattataatcctccgtggacgttcggccaagggaccaaggtagcaatcaag

SEQ ID NO: 64 - DNA, 339 bp, Artificial Sequence
  source: /note="Description of Artificial Sequence: Synthetic polynucleotide"
gacatcgtgatgacccagtctccaaactccctggctgtgtctctgggcgggagggccaccatcaactgcaagaccagccagagtattttatacaggtccaacaataagaactacttagcttggtaccagcataaaccaggacagcctcccaagctgctcatttactgggcatctacccgggaatccagggtccctgaccgattcagtggcagcgggtctaggacagatttcactctcaccatcagcggcctgcaggctgaagatgtggcagtttattactgtcagcaatattataatcctccgtggacgttcggccaggggaccaaggtggaaatcaaa

SEQ ID NO: 65 - DNA, 339 bp, Artificial Sequence
  source: /note="Description of Artificial Sequence: Synthetic polynucleotide"
gacatcgtgatgacccagtctccaaactccctggctgtgtctctgggcgggagggccaccatcaactgcaagaccagccagagtattttatacaggtccaacaataagaactacttagcttggtaccagcataaatcaggacagcctcccaagctgctcatttactgggcatctacccgggaatccggggtccctgaccgattcagtggcagcgggtctaggacagatttcactctcaccatcagcggcctgcaggctgaagatgtggcagtttattactgtcagcaatattataatcctccgtggacgttcggccaagggaccaaggtggaaatcaaa

SEQ ID NO: 66 - DNA, 339 bp, Artificial Sequence; identical to SEQ ID NO: 65
  source: /note="Description of Artificial Sequence: Synthetic polynucleotide"

SEQ ID NO: 67 - DNA, 339 bp, Artificial Sequence
  source: /note="Description of Artificial Sequence: Synthetic polynucleotide"
gacatcgtgatgacccagtctccggactccctgactgtgtctctgggcgagagggccaccatcagctgcaagtccagccagcgtcttttgtatagttccaacaataagaactacttagcttggtaccagcagaaacctggacagcctcctaaactgctcatgtactgggcgtccacccgggaatccggggtccctgaccgattcagtggcagcgggtctgggacagatttctctctcaccatcagcagcctgcaggctgaagatgtggcagtttattactgtcagcaatattataatcctccctggacgttcggccaagggaccaaggtggaagtcaaa

SEQ ID NO: 68 - DNA, 339 bp, Artificial Sequence; identical to SEQ ID NO: 67
  source: /note="Description of Artificial Sequence: Synthetic polynucleotide"

SEQ ID NO: 69 - DNA, 339 bp, Artificial Sequence
  source: /note="Description of Artificial Sequence: Synthetic polynucleotide"
gacatcgtgatgacccagtctccagattccctgactctgtctctgggcgagagggccaccatcaactgcaagtccagccagagtctgttttacaggtccaacaataagagctacttagcttggtatcagcaaaaaccagggcagcctcctaaactgctcatttactgggcctctgtccgggaatccggggtccctgaccgattcactggcagcgggtctgtaacagatttcactctcaccatcagcagcctgcgggctgaggatgtggctgtttattattgtcaacagtattttactactcctctcactttcggcggggggaccaaggtggcgatcaaa

SEQ ID NO: 70 - DNA, 339 bp, Artificial Sequence
  source: /note="Description of Artificial Sequence: Synthetic polynucleotide"
gacatcgtgatgacccagtctctagactccctgactgtgtctctgggcgagagggccaccatcaactgcaagtccagccagagtcttttatacacctccaacaataagaattacttagcttggtaccagcagaaatcaggacagcctcctaagttactcatttactgggcgtctattcgggattccggggtccctgaccgattcagtggcagcgggtctgcgacagatttcactctcaccatcaacaacctgcaggctgaagatgtggcagtttacttctgtcagcaatattacaagactcctctcactttcggcggggggaccaaggtggaggtcaga

SEQ ID NO: 71 - DNA, 321 bp, Artificial Sequence
  source: /note="Description of Artificial Sequence: Synthetic polynucleotide"
gacatccagwtgacccagtctccttccaccctgtctgcatctgtaggagacagagtcaccatcacttgccgggccagtcagagtattagtagctggttggcctggtatcagcagaaaccagggaaagcccctaagctcctgatctataaggcgtctagtttagaaagtggggtcccatcaaggttcagcggcagtggatctgggacagaattcactctcaccatcagcagcctgcagcctgatgattttgcaacttattactgccaacagtataatagttattcttggacgttcggccaagggaccaaggtggaaatcaaa

SEQ ID NO: 72 - protein, 120 aa, Artificial Sequence; identical to SEQ ID NO: 4
  source: /note="Description of Artificial Sequence: Synthetic polypeptide"

SEQ ID NO: 73 - protein, 116 aa, Artificial Sequence; identical to SEQ ID NO: 5
  source: /note="Description of Artificial Sequence: Synthetic polypeptide"

SEQ ID NO: 74 - protein, 116 aa, Artificial Sequence; identical to SEQ ID NO: 6
  source: /note="Description of Artificial Sequence: Synthetic polypeptide"

SEQ ID NO: 75 - protein, 116 aa, Artificial Sequence; identical to SEQ ID NO: 10
  source: /note="Description of Artificial Sequence: Synthetic polypeptide"

SEQ ID NO: 76 - protein, 116 aa, Artificial Sequence; identical to SEQ ID NO: 12
  source: /note="Description of Artificial Sequence: Synthetic polypeptide"

SEQ ID NO: 77 - protein, 116 aa, Artificial Sequence; identical to SEQ ID NO: 13
  source: /note="Description of Artificial Sequence: Synthetic polypeptide"

SEQ ID NO: 78 - protein, 116 aa, Artificial Sequence; identical to SEQ ID NO: 14
  source: /note="Description of Artificial Sequence: Synthetic polypeptide"

SEQ ID NO: 79 - protein, 116 aa, Artificial Sequence; identical to SEQ ID NO: 16
  source: /note="Description of Artificial Sequence: Synthetic polypeptide"

SEQ ID NO: 80 - protein, 121 aa, Artificial Sequence; identical to SEQ ID NO: 18
  source: /note="Description of Artificial Sequence: Synthetic polypeptide"

SEQ ID NO: 81 - protein, 118 aa, Artificial Sequence; identical to SEQ ID NO: 19
  source: /note="Description of Artificial Sequence: Synthetic polypeptide"

SEQ ID NO: 82 - protein, 124 aa, Artificial Sequence; identical to SEQ ID NO: 20
  source: /note="Description of Artificial Sequence: Synthetic polypeptide"

SEQ ID NO: 83 - protein, 110 aa, Artificial Sequence; identical to SEQ ID NO: 21
  source: /note="Description of Artificial Sequence: Synthetic polypeptide"

SEQ ID NO: 84 - protein, 110 aa, Artificial Sequence; identical to SEQ ID NO: 22
  source: /note="Description of Artificial Sequence: Synthetic polypeptide"

SEQ ID NO: 85 - protein, 110 aa, Artificial Sequence; identical to SEQ ID NO: 27
  source: /note="Description of Artificial Sequence: Synthetic polypeptide"

SEQ ID NO: 86 - protein, 110 aa, Artificial Sequence; identical to SEQ ID NO: 29
  source: /note="Description of Artificial Sequence: Synthetic polypeptide"

SEQ ID NO: 87 - protein, 110 aa, Artificial Sequence; identical to SEQ ID NO: 30
  source: /note="Description of Artificial Sequence: Synthetic polypeptide"

SEQ ID NO: 88 - protein, 110 aa, Artificial Sequence; identical to SEQ ID NO: 31
  source: /note="Description of Artificial Sequence: Synthetic polypeptide"

SEQ ID NO: 89 - protein, 110 aa, Artificial Sequence; identical to SEQ ID NO: 33
  source: /note="Description of Artificial Sequence: Synthetic polypeptide"

SEQ ID NO: 90 - protein, 113 aa, Artificial Sequence; identical to SEQ ID NO: 35
  source: /note="Description of Artificial Sequence: Synthetic polypeptide"

SEQ ID NO: 91 - protein, 110 aa, Artificial Sequence; identical to SEQ ID NO: 36
  source: /note="Description of Artificial Sequence: Synthetic polypeptide"

SEQ ID NO: 92 - protein, 107 aa, Artificial Sequence; identical to SEQ ID NO: 37
  source: /note="Description of Artificial Sequence: Synthetic polypeptide"
  MOD_RES (4)..(4): Any amino acid

SEQ ID NO: 93 - DNA, 369 bp, Artificial Sequence
  source: /note="Description of Artificial Sequence: Synthetic polynucleotide"
gaggtgcagctggtggagtctgggggaggcgtggtccagcctgggaggtccctgagactctcctgcgcagcctctggactcaccttcagtttctataatttccactgggtccgccagactccaggcaaggggctggagtgggtggcaggcatctcatacgatgcaaccaggacgaactacgcaggctccgtgacgggccgattcaccatttccagagacaattccaagaaaatgctgtatctgcaaatgagcagcctgggacctcaagacacggctgtatatcattgtgcgagagatcgttctgacgggcaactgcataaagtggcttttgactcctggggccagggagccctggtcaccgtctcatca

SEQ ID NO: 94 - DNA, 357 bp, Artificial Sequence; identical to SEQ ID NO: 39
  source: /note="Description of Artificial Sequence: Synthetic polynucleotide"

SEQ ID NO: 95 - DNA, 357 bp, Artificial Sequence; identical to SEQ ID NO: 40
  source: /note="Description of Artificial Sequence: Synthetic polynucleotide"

SEQ ID NO: 96 - DNA, 357 bp, Artificial Sequence; identical to SEQ ID NO: 45
  source: /note="Description of Artificial Sequence: Synthetic polynucleotide"

SEQ ID NO: 97 - DNA, 357 bp, Artificial Sequence; identical to SEQ ID NO: 46
  source: /note="Description of Artificial Sequence: Synthetic polynucleotide"

SEQ ID NO: 98 - DNA, 357 bp, Artificial Sequence; identical to SEQ ID NO: 47
  source: /note="Description of Artificial Sequence: Synthetic polynucleotide"

SEQ ID NO: 99 - DNA, 357 bp, Artificial Sequence; identical to SEQ ID NO: 48
  source: /note="Description of Artificial Sequence: Synthetic polynucleotide"

SEQ ID NO: 100 - DNA, 357 bp, Artificial Sequence; identical to SEQ ID NO: 51
  source: /note="Description of Artificial Sequence: Synthetic polynucleotide"

SEQ ID NO: 101 - DNA, 363 bp, Artificial Sequence; identical to SEQ ID NO: 52
  source: /note="Description of Artificial Sequence: Synthetic polynucleotide"

SEQ ID NO: 102 - DNA, 363 bp, Artificial Sequence; identical to SEQ ID NO: 53
  source: /note="Description of Artificial Sequence: Synthetic polynucleotide"

SEQ ID NO: 103 - DNA, 372 bp, Artificial Sequence; identical to SEQ ID NO: 54
  source: /note="Description of Artificial Sequence: Synthetic polynucleotide"

SEQ ID NO: 104 - DNA, 339 bp, Artificial Sequence; identical to SEQ ID NO: 55
  source: /note="Description of Artificial Sequence: Synthetic polynucleotide"

SEQ ID NO: 105 - DNA, 339 bp, Artificial Sequence
  source: /note="Description of Artificial Sequence: Synthetic polynucleotide"
gacatcgtgatgacccagtctccaggctccctggctgtgtctctgggctcgagggccaccatcaactgcaagtccagccggagtcttttatacaggtccaacaataagaattatttagcttggtatcaacagaaaccaggacagtctcctcggcttctcatttattgggcatcttcccgggaatccggggtccctgaccgattcagtggcggcgggtctgggacaagtttcactctcaccatcagcagcctgcaggctgaagatgtggcagtttattactgtcagcaatattttaatcctccgtggacgttcggccaagggaccaaggtggagatcaaa

SEQ ID NO: 106 - DNA, 339 bp, Artificial Sequence; identical to SEQ ID NO: 61
  source: /note="Description of Artificial Sequence: Synthetic polynucleotide"

SEQ ID NO: 107 - DNA, 339 bp, Artificial Sequence; identical to SEQ ID NO: 63
  source: /note="Description of Artificial Sequence: Synthetic polynucleotide"

SEQ ID NO: 108 - DNA, 339 bp, Artificial Sequence; identical to SEQ ID NO: 64
  source: /note="Description of Artificial Sequence: Synthetic polynucleotide"

SEQ ID NO: 109 - DNA, 339 bp, Artificial Sequence; identical to SEQ ID NO: 65
  source: /note="Description of Artificial Sequence: Synthetic polynucleotide"

SEQ ID NO: 110 - DNA, 339 bp, Artificial Sequence; identical to SEQ ID NO: 67
  source: /note="Description of Artificial Sequence: Synthetic polynucleotide"

SEQ ID NO: 111 - DNA, 339 bp, Artificial Sequence; identical to SEQ ID NO: 69
  source: /note="Description of Artificial Sequence: Synthetic polynucleotide"

SEQ ID NO: 112 - DNA, 339 bp, Artificial Sequence; identical to SEQ ID NO: 70
  source: /note="Description of Artificial Sequence: Synthetic polynucleotide"

SEQ ID NO: 113 - DNA, 321 bp, Artificial Sequence; identical to SEQ ID NO: 71
  source: /note="Description of Artificial Sequence: Synthetic polynucleotide"

SEQ ID NO: 114 - protein, 15 aa, Homo sapiens
GPPPPIDNGDITSFP

SEQ ID NO: 115 - protein, 19 aa, Artificial Sequence
  source: /note="Description of Artificial Sequence: Synthetic peptide"
  source: /note="C-term Biotin"
GPPPPIDNGDITSFPGGGK

SEQ ID NO: 116 - protein, 6 aa, Artificial Sequence
  source: /note="Description of Artificial Sequence: Synthetic 6xHis tag"
HHHHHH

SEQ ID NO: 117 - protein, 5 aa, Unknown
  source: /note="Description of Unknown: Enterokinase cleavage site sequence"
DDDDK

SEQ ID NO: 118 - protein, 6 aa, Unknown
  source: /note="Description of Unknown: Enterokinase cleavage site sequence"
ADDDDK

SEQ ID NO: 119 - skipped

SEQ ID NO: 120 - protein, 12 aa, Artificial Sequence
  source: /note="Description of Artificial Sequence: Synthetic peptide"
  source: /note="C-term Biotin"
PIDNGDITGGGK

SEQ ID NO: 121 - protein, 15 aa, Homo sapiens
EFGKCGPPPPIDNGD

SEQ ID NO: 122 - protein, 15 aa, Homo sapiens
FGKCGPPPPIDNGDI

SEQ ID NO: 123 - protein, 15 aa, Homo sapiens
GKCGPPPPIDNGDIT

SEQ ID NO: 124 - protein, 15 aa, Homo sapiens
KCGPPPPIDNGDITS

SEQ ID NO: 125 - protein, 15 aa, Homo sapiens
CGPPPPIDNGDITSF

SEQ ID NO: 126 - protein, 15 aa, Homo sapiens
GPPPPIDNGDITSFP

SEQ ID NO: 127 - protein, 15 aa, Homo sapiens
PPPPIDNGDITSFPL

SEQ ID NO: 128 - protein, 15 aa, Homo sapiens
PPPIDNGDITSFPLS

SEQ ID NO: 129 - protein, 15 aa, Homo sapiens
PPIDNGDITSFPLSV

SEQ ID NO: 130 - protein, 15 aa, Homo sapiens
PIDNGDITSFPLSVY

SEQ ID NO: 131 - protein, 15 aa, Homo sapiens
IDNGDITSFPLSVYA

SEQ ID NO: 132 - protein, 15 aa, Homo sapiens
DNGDITSFPLSVYAP